European Patent Application EP 4 269 618 A2, published November 1, 2023. Title: HIGH-THROUGHPUT SINGLE-CELL TRANSCRIPTOME LIBRARIES AND METHODS OF MAKING AND OF USING. Applicant: ILLUMINA, INC. Application WO PCT/US2019/035422, filed June 4, 2019. The sequence listing filed with the application follows.

SEQUENCE LISTING (14 sequences)

SEQ ID NO: 1 - DNA, 54 bp, synthetic construct
  misc_feature 1..54: note = Description of Artificial Sequence: Synthetic primer
  modified_base 7..24: mod_base = OTHER; note = a, c, t, g, unknown or other
  source 1..54: mol_type = other DNA
cagagcnnnnnnnnnnnnnnnnnntttttttttttttttttttttttttttttt

SEQ ID NO: 2 - DNA, 45 bp, synthetic construct
  misc_feature 1..45: note = Description of Artificial Sequence: Synthetic oligonucleotide
  misc_feature 1..45: note = Description of Combined DNA/RNA Molecule: Synthetic oligonucleotide
  modified_base 7..16: mod_base = OTHER; note = a, c, t, g, unknown or other
  modified_base 36..45: mod_base = OTHER; note = a, c, t, g, unknown or other
  source 1..45: mol_type = other DNA
  modified_base 17: mod_base = OTHER; note = ideoxyU
  misc_feature 1..16: note = DNA
  misc_feature 17: note = RNA
  misc_feature 18..45: note = DNA
gctctgnnnnnnnnnntacgacgctcttccgatctnnnnnnnnnn

SEQ ID NO: 3 - DNA, 29 bp, synthetic construct
  misc_feature 1..29: note = Description of Artificial Sequence: Synthetic primer
  source 1..29: mol_type = other DNA
aatgatacggcgaccaccgagatctacac

SEQ ID NO: 4 - DNA, 24 bp, synthetic construct
  misc_feature 1..24: note = Description of Artificial Sequence: Synthetic primer
  source 1..24: mol_type = other DNA
caagcagaagacggcatacgagat

SEQ ID NO: 5 - DNA, 68 bp, synthetic construct
  misc_feature 1..68: note = Description of Artificial Sequence: Synthetic primer
  modified_base 19..36: mod_base = OTHER; note = a, c, t, g, unknown or other
  modified_base 68: mod_base = OTHER; note = a, c, t, g, unknown or other
  source 1..68: mol_type = other DNA
acgacgctcttccgatctnnnnnnnnnnnnnnnnnnttttttttttttttttttttttttttttttvn

SEQ ID NO: 6 - DNA, 29 bp, synthetic construct
  misc_feature 1..29: note = Description of Artificial Sequence: Synthetic primer
  source 1..29: mol_type = other DNA
aatgatacggcgaccaccgagatctacac

SEQ ID NO: 7 - DNA, 24 bp, synthetic construct
  misc_feature 1..24: note = Description of Artificial Sequence: Synthetic primer
  source 1..24: mol_type = other DNA
caagcagaagacggcatacgagat

SEQ ID NO: 8 - DNA, 33 bp, synthetic construct
  misc_feature 1..33: note = Description of Artificial Sequence: Synthetic primer
  source 1..33: mol_type = other DNA
acactctttccctacacgacgctcttccgatct

SEQ ID NO: 9 - DNA, 15 bp, synthetic construct
  misc_feature 1..15: note = Description of Artificial Sequence: Synthetic primer
  source 1..15: mol_type = other DNA
gtctcgtgggctcgg

SEQ ID NO: 10 - DNA, 33 bp, synthetic construct; identical to SEQ ID NO: 8
  misc_feature 1..33: note = Description of Artificial Sequence: Synthetic primer
  source 1..33: mol_type = other DNA

SEQ ID NO: 11 - DNA, 15 bp, synthetic construct
  misc_feature 1..15: note = Description of Artificial Sequence: Synthetic primer
  source 1..15: mol_type = other DNA
gtctcgtgggctcgg

SEQ ID NO: 12 - DNA, 44 bp, synthetic construct
  misc_feature 1..15: note = DNA
  source 1..44: mol_type = other DNA
  misc_feature 1..44: note = Description of Combined DNA/RNA Molecule: Synthetic oligonucleotide
  modified_base 7..15: mod_base = OTHER; note = a, c, t, g, unknown or other
  modified_base 35..44: mod_base = OTHER; note = a, c, t, g, unknown or other
  misc_feature 1..44: note = Description of Artificial Sequence: Synthetic oligonucleotide
  misc_feature 16: note = RNA
  misc_feature 17..44: note = DNA
gctctgnnnnnnnnntacgacgctcttccgatctnnnnnnnnnn

SEQ ID NO: 13 - DNA, 43 bp, synthetic construct
  misc_feature 1..15: note = DNA
  source 1..43: mol_type = other DNA
  modified_base 7..15: mod_base = OTHER; note = a, c, t, g, unknown or other
  modified_base 35..43: mod_base = OTHER; note = a, c, t, g, unknown or other
  misc_feature 1..43: note = Description of Combined DNA/RNA Molecule: Synthetic oligonucleotide
  misc_feature 1..43: note = Description of Artificial Sequence: Synthetic oligonucleotide
  misc_feature 16: note = RNA
  misc_feature 17..43: note = DNA
gctctgnnnnnnnnntacgacgctcttccgatctnnnnnnnnn

SEQ ID NO: 14 - DNA, 44 bp, synthetic construct
  source 1..44: mol_type = other DNA
  modified_base 7..16: mod_base = OTHER; note = a, c, t, g, unknown or other
  modified_base 36..44: mod_base = OTHER; note = a,c, t, g, unknown or other
  misc_feature 1..44: note = Description of Combined DNA/RNA Molecule: synthetic oligonucleotide
  misc_feature 1..44: note = Description of Artificial Sequence: Synthetic oligonucleotide
  misc_feature 1..16: note = DNA
  misc_feature 17: note = RNA
  misc_feature 18..44: note = DNA
gctctgnnnnnnnnnntacgacgctcttccgatctnnnnnnnnn